European Patent Application EP 4 585 698 A2, published July 16, 2025. Title: Zastosowanie polimerazy TaqNeqSSB do normalizacji temperatury przyłączania sond i starterów w reakcji wykrywania jednonukleotydowych mutacji SNP. Applicant: Instytut Biotechnologii i Medycyny Molekularnej. Application PL, filed December 23, 2023. The sequence listing filed with the application follows.

SEQUENCE LISTING (60 sequences)

SEQ ID NO: 1 - DNA, 277 bp, Homo sapiens
  source 1..277: mol_type = other DNA
aataagtacatcttattaactgatttgacctgaggcactttgaggggtcctgttgtaatcttgccactttcctctgcttttctcatttatccctctttttttgcaacttgagaagtaaaacagcagcctaccaaggtgaggccacagttgcagngataacatttgagccaaggcttcataagggctgctgtaggaggggagagcatcctggcactttagtgggctacgtggccgactgcaattgcaaggattagcagtgtgagccctgatcctgcta

SEQ ID NO: 2 - DNA, 220 bp, Homo sapiens
  source 1..220: mol_type = other DNA
tagatggcagtcaccttagcaataagccatcctggaagtgaatcctctaacctcagtccctccagttgctgtcacacatantagagatgaagccttcagccaagtcctgtccaagttcctgacctataaaatcttgagcaaaatagagtactgtagttattttaaatcattcagctttgggttagcttgttatgcaacaacaataatcaaaacacagggt

SEQ ID NO: 3 - DNA, 326 bp, Homo sapiens
  source 1..326: mol_type = other DNA
gctttggattccagctcaaggagggtctgcaggttacagtgagggcccgaaactcagaaagcgagggggcctgcccagcagtctggcccgcggagccctcccagctgcccatggattgcatcactgtcccaaggggagacagggctgtcctgccggctgcctctttgagtcaccntgtggccagggagtcctgctggcctccacagtcaccgccaaaccattttggccttggtctttcaaagccaggtcattttgggaaaactgaggacatccagcaccatggaggggcgtgtgtgtctctgcactggctgatgaagggaggtggg

SEQ ID NO: 4 - DNA, 383 bp, Homo sapiens
  source 1..383: mol_type = other DNA
ctaagtgaacactgccttcccattgatgaccttgagaggttagagaccaatggcagtgacggtgatcacattattatttgaagccttatttgaatatttaagacttagtatgtttgtttaaaaaaataatcatgttgcatcataaccatactttgtaagaccagattaccggtgaccgctcgngatgttaagctagtgaagacaatgcaaggtggcctgaagcagcatgaggcagaccatggtcccgacctgcattggctggtgctggctgcagctgctgatggaggctacaaacagtgatagaagcatgcagaagctacacagcacaggccaaggtgctgtgggagaggcggaggaggaacactgaccactggcggcctggg

SEQ ID NO: 5 - DNA, 214 bp, Homo sapiens
  source 1..214: mol_type = other DNA
ggtgcagaccacaggccaggactgtgctaaagnctacacttggcttattgccctcagtcctcaaaacagccctgtgcagtaggcattgtagttgaccttgtcttacaggtggggagaatgagccacagagaaaataaataatttctgggaaatcatccaacaagcaaatggtattgctgggattttgagtccatcctgccaccagcttccaggc

SEQ ID NO: 6 - DNA, 270 bp, Homo sapiens
  source 1..270: mol_type = other DNA
tgttactaccataatggcttatgtggtttataatgcctcttaaatgaacacaatatcagtctgcaaccaggcagcaaggtttgggatganatcattgtcacagggtagagaggctgctggaatccaactcatggctcaactggactaacaacacacaccagaaacattcttaccttctgcctcatgcttcagagagctttaagcaccaggtgtaggtgtgataaggaatgcgattagtggtatttattaaatgaaatattgtctatggat

SEQ ID NO: 7 - DNA, 270 bp, Homo sapiens
  source 1..270: mol_type = other DNA
agagaacagaggattcccttccagggaaacacaccaacataaaaggaaaaacaaaaacaaacaaaaaactaccaatactaataggngattgctgtattccagagttccagatccctgcctaatcaacctacaatgaagtttctattcagccaggtcagaccatgtgcacagagcttccagtgatcactttagtgcctcactcttaaatgtgaccagacaacctgggatcaccaaacatttgaagaaatcctctaacatgattaatgatta

SEQ ID NO: 8 - DNA, 270 bp, Homo sapiens
  source 1..270: mol_type = other DNA
atgtcttatatctctctttctcatcccagaggcaatcgctctattgaaatttgttttcattgttattgtcctttttacaaatacctctanactttcccacaatccacacacagtattgttttacatgttttgtaaatgtgcataaatgacatgtccttggtgtcaattcagatttccttttgggtcagtacttttgtgaaattcatacatatcgaggcttatagatcaatttcatatactatcattactgttaaatccagcatctgcata

SEQ ID NO: 9 - DNA, 221 bp, Homo sapiens
  source 1..221: mol_type = other DNA
taaaaggaaagttaccaaaataatcacatagcagatcatcaacccaatacataaccctagaaatgaaaattgccccagctgtgcctatccatccagcatgttccagtcctatactcctacatctcttatttctccacttttttcacggttctctgcttaaatgtgcacacactggagaggacctttttgaataccttaaatgaacttgttgtacaaatgta

SEQ ID NO: 10 - DNA, 270 bp, Homo sapiens
  source 1..270: mol_type = other DNA
ccatgtctacatgtcgcctaaagtcatgtcacacaccacattcatcccacactttgggaaactcgcagcaccatgtcatcacttgctnaatagaatccagtcgtggcttttcaggggacactgagacacgcaaaacctgtcaggctgatgagccaaggacgtttccagtggtttcgcaagcctcctccaagtgttgatggctgccagctttcctcatctggcctctcgtagcaaattaacttagtcaacattcacttacacaaatatttg

SEQ ID NO: 11 - DNA, 270 bp, Homo sapiens
  source 1..270: mol_type = other DNA
gaaggatgctgcttttgaatgaaacccagagcaagagatacctctagagcagattcaggctgcaatacaatccccactgccagngagtcacatgacagaggactggaggtatctgtagcaatcaagatgtggttgcatcttaggcaagtcctaacagaagagtctcagagaataaccctggggttttgcagcaagtccgtgtcctcttgtgttagtctgctggggctgctattacaaaataccacagactgggtattaaacaacaaaaca

SEQ ID NO: 12 - DNA, 270 bp, Homo sapiens
  source 1..270: mol_type = other DNA
cagtagaggcggcatttgaggcgctgacccatgacaggaggagcacgggctacagccgaggacacactgctagcagccataacngtggcaagtgttgaacaagcagaaaagatgtaatagttgtgaagtcagaggagtagtcagcgacattggcctgggtccttccgtgaggagcagactcgaatgctaaaatacactcccatgcctcttcccacagcactgccaccacctagaattaaatttttgacagtaacagcaatcgcgtgtttt

SEQ ID NO: 13 - DNA, 21 bp, Homo sapiens
  source 1..21: mol_type = other DNA
catggtatcagacgctggctc

SEQ ID NO: 14 - DNA, 21 bp, Homo sapiens
  source 1..21: mol_type = other DNA
catggtatcagacgctggctc

SEQ ID NO: 15 - DNA, 21 bp, Homo sapiens
  source 1..21: mol_type = other DNA
gtgcctcaggtcaaatcagtt

SEQ ID NO: 16 - DNA, 27 bp, Homo sapiens
  source 1..27: mol_type = other DNA
cttgctttgcaggttgcacgagaccta

SEQ ID NO: 17 - DNA, 28 bp, Homo sapiens
  source 1..28: mol_type = other DNA
acttgctttgcagtttgcacgagaccta

SEQ ID NO: 18 - DNA, 21 bp, Homo sapiens
  source 1..21: mol_type = other DNA
aggaggacacagagagaccaa

SEQ ID NO: 19 - DNA, 21 bp, Homo sapiens
  source 1..21: mol_type = other DNA
aacttggacaggacttggctg

SEQ ID NO: 20 - DNA, 32 bp, Homo sapiens
  source 1..32: mol_type = other DNA
ccagttgctgtcacacatattagagatgaagc

SEQ ID NO: 21 - DNA, 31 bp, Homo sapiens
  source 1..31: mol_type = other DNA
ccagttgctgtcacacatactagagatgaag

SEQ ID NO: 22 - DNA, 21 bp, Homo sapiens
  source 1..21: mol_type = other DNA
aaatggtttggcggtgactgt

SEQ ID NO: 23 - DNA, 25 bp, Homo sapiens
  source 1..25: mol_type = other DNA
ccacacggtgactcaaagaggcagc

SEQ ID NO: 24 - DNA, 25 bp, Homo sapiens
  source 1..25: mol_type = other DNA
ccacatggtgactcaaagaggcagc

SEQ ID NO: 25 - DNA, 24 bp, Homo sapiens
  source 1..24: mol_type = other DNA
tgttgcatcataaccatactttgt

SEQ ID NO: 26 - DNA, 19 bp, Homo sapiens
  source 1..19: mol_type = other DNA
cttcaggccaccttgcatt

SEQ ID NO: 27 - DNA, 30 bp, Homo sapiens
  source 1..30: mol_type = other DNA
cttcactagcttaacatcacgagcggtcac

SEQ ID NO: 28 - DNA, 30 bp, Homo sapiens
  source 1..30: mol_type = other DNA
cttcactagcttaacatcccgagcggtcac

SEQ ID NO: 29 - DNA, 21 bp, Homo sapiens
  source 1..21: mol_type = other DNA
cagctcccagttcataccagg

SEQ ID NO: 30 - DNA, 21 bp, Homo sapiens
  source 1..21: mol_type = other DNA
ctgttttgaggactgagggca

SEQ ID NO: 31 - DNA, 25 bp, Homo sapiens
  source 1..25: mol_type = other DNA
ccaggactgtgctaaaggctacact

SEQ ID NO: 32 - DNA, 25 bp, Homo sapiens
  source 1..25: mol_type = other DNA
ccaggactgtgctaaagactacact

SEQ ID NO: 33 - DNA, 23 bp, Homo sapiens
  source 1..23: mol_type = other DNA
aacacaatatcagtctgcaacca

SEQ ID NO: 34 - DNA, 21 bp, Homo sapiens
  source 1..21: mol_type = other DNA
tccagttgagccatgagttgg

SEQ ID NO: 35 - DNA, 29 bp, Homo sapiens
  source 1..29: mol_type = other DNA
cctctctaccctgtgacaatgatctcatc

SEQ ID NO: 36 - DNA, 29 bp, Homo sapiens
  source 1..29: mol_type = other DNA
cctctctaccctgtgacaatgatttcatc

SEQ ID NO: 37 - DNA, 21 bp, Homo sapiens
  source 1..21: mol_type = other DNA
tcaggcaagagaacagaggat

SEQ ID NO: 38 - DNA, 24 bp, Homo sapiens
  source 1..24: mol_type = other DNA
aacttcattgtaggttgattaggc

SEQ ID NO: 39 - DNA, 32 bp, Homo sapiens
  source 1..32: mol_type = other DNA
atctggaactctggaatacagcaatcacctat

SEQ ID NO: 40 - DNA, 32 bp, Homo sapiens
  source 1..32: mol_type = other DNA
atctggaactctggaatacagcaatcgcctat

SEQ ID NO: 41 - DNA, 21 bp, Homo sapiens
  source 1..21: mol_type = other DNA
ccagaggcaatcgctctattg

SEQ ID NO: 42 - DNA, 25 bp, Homo sapiens
  source 1..25: mol_type = other DNA
aatctgaattgacaccaaggacatg

SEQ ID NO: 43 - DNA, 33 bp, Homo sapiens
  source 1..33: mol_type = other DNA
tacctctatactttcccacaatccacacacagt

SEQ ID NO: 44 - DNA, 33 bp, Homo sapiens
  source 1..33: mol_type = other DNA
tacctctacactttcccacaatccacacacagt

SEQ ID NO: 45 - DNA, 22 bp, Homo sapiens
  source 1..22: mol_type = other DNA
tcacatagcagatcatcaaccc

SEQ ID NO: 46 - DNA, 21 bp, Homo sapiens
  source 1..21: mol_type = other DNA
aaaggtcctctccagtgtgtg

SEQ ID NO: 47 - DNA, 28 bp, Homo sapiens
  source 1..28: mol_type = other DNA
tgtgcctatcatccagcatgttccagtc

SEQ ID NO: 48 - DNA, 28 bp, Homo sp.
  source 1..28: mol_type = other DNA
tgtgcctaccatccagcatgttccagtc

SEQ ID NO: 49 - DNA, 22 bp, Homo sapiens
  source 1..22: mol_type = other DNA
gtcgcctaaagtcatgtcacac

SEQ ID NO: 50 - DNA, 22 bp, Homo sapiens
  source 1..22: mol_type = other DNA
tggaaacgtccttggctcatca

SEQ ID NO: 51 - DNA, 34 bp, Homo sapiens
  source 1..34: mol_type = other DNA
atgtcatcacttgctaaatagaatccagtcgtgg

SEQ ID NO: 52 - DNA, 34 bp, Homo sapiens
  source 1..34: mol_type = other DNA
atgtcatcacttgctgaatagaatccagtcgtgg

SEQ ID NO: 53 - DNA, 21 bp, Homo sapiens
  source 1..21: mol_type = other DNA
gctgcttttgaatgaaaccca

SEQ ID NO: 54 - DNA, 22 bp, Homo sapiens
  source 1..22: mol_type = other DNA
accacatcttgattgctacaga

SEQ ID NO: 55 - DNA, 26 bp, Homo sapiens
  source 1..26: mol_type = other DNA
tcctctgtcatgtgactcactggcag

SEQ ID NO: 56 - DNA, 26 bp, Homo sapiens
  source 1..26: mol_type = other DNA
tcctctgtcatgtgactcgctggcag

SEQ ID NO: 57 - DNA, 20 bp, Homo sapiens
  source 1..20: mol_type = other DNA
gtcagtagaggcggcatttg

SEQ ID NO: 58 - DNA, 20 bp, Homo sapiens
  source 1..20: mol_type = other DNA
tcgctgactactcctctgac

SEQ ID NO: 59 - DNA, 28 bp, Homo sapiens
  source 1..28: mol_type = other DNA
ccataacggtggcaagtgttgaacaagc

SEQ ID NO: 60 - DNA, 28 bp, Homo sapiens
  source 1..28: mol_type = other DNA
ccataacagtggcaagtgttgaacaagc